European Patent Application EP 4 644 422 A1, published November 5, 2025. Title: ANTI-NKG2A ANTIBODY AND USE THEREOF. Applicant: BioRay Pharmaceutical Co., Ltd. Application EP. The sequence listing filed with the application follows.

SEQUENCE LISTING (167 sequences)

SEQ ID NO: 1 - protein, 121 aa, synthetic construct
EVQLQQSVAELVRPGASVKLSCTASGFNIQNTYMHWVKERPEQGLEWIGRIDPANGDTEFAPKFQGKATLTTDTSSNTAYLQLSSLTSEDTAIYYCGRERYFYGSRGFAYWGQGTLVTVSA

SEQ ID NO: 2 - protein, 5 aa, synthetic construct
NTYMH

SEQ ID NO: 3 - protein, 17 aa, synthetic construct
RIDPANGDTEFAPKFQG

SEQ ID NO: 4 - protein, 12 aa, synthetic construct
ERYFYGSRGFAY

SEQ ID NO: 5 - protein, 107 aa, synthetic construct
DILMTQSPPSMSVSLGDTVSITCHASQGISSNIGWLQQKPGKSFKGLIYHGTNLEDGVPSRFSGSGSGADYSLTISSLESEDFADYYCVQYAQFPWTFGGGTKLEIK

SEQ ID NO: 6 - protein, 11 aa, synthetic construct
HASQGISSNIG

SEQ ID NO: 7 - protein, 7 aa, synthetic construct
HGTNLED

SEQ ID NO: 8 - protein, 9 aa, synthetic construct
VQYAQFPWT

SEQ ID NO: 9 - protein, 122 aa, synthetic construct
EVQLQQSVAELVRPGASVKLSCTASGFNIKNTYIHWVKQRPEQGLEWIGRIDPANGNTKYAPKFQGKASIIVDTSSNTAYLQLSSLTSEDTAIYYCARYYASSPYYYNMDYWGQGTSVTVSS

SEQ ID NO: 10 - protein, 5 aa, synthetic construct
NTYIH

SEQ ID NO: 11 - protein, 17 aa, synthetic construct
RIDPANGNTKYAPKFQG

SEQ ID NO: 12 - protein, 13 aa, synthetic construct
YYASSPYYYNMDY

SEQ ID NO: 13 - protein, 106 aa, synthetic construct
DIQMTQSPASLSVSVGETVTITCRASENIYSNLAWYQQKQGKSPQLLVYAATNLADGVPSRFSGSGSGTQYSLKINSLQSEDFGSYYCQHFWGTFTFGSGTKLEIK

SEQ ID NO: 14 - protein, 11 aa, synthetic construct
RASENIYSNLA

SEQ ID NO: 15 - protein, 7 aa, synthetic construct
AATNLAD

SEQ ID NO: 16 - protein, 8 aa, synthetic construct
QHFWGTFT

SEQ ID NO: 17 - protein, 119 aa, synthetic construct
EVQLQQSVAELVRPGASVKLSCTASGFNIKNTYIDWVKQRPEQGLEWIGNIDPANGNTKYAPKFQGKATITADTSSNTAYVQLSSLTSEDTAIYYCARWGGWDVRFAYWGQGTLVTVSA

SEQ ID NO: 18 - protein, 5 aa, synthetic construct
NTYID

SEQ ID NO: 19 - protein, 17 aa, synthetic construct
NIDPANGNTKYAPKFQG

SEQ ID NO: 20 - protein, 10 aa, synthetic construct
WGGWDVRFAY

SEQ ID NO: 21 - protein, 107 aa, synthetic construct
DIKMTQSPSSMYASLGERVTITCKASQDINTYLSWFQQKPGKSPKTLIYRANRLVDGVPSRFSGSGSGQNYSLTISSLEYEDMGIYYCLQYDEFPLTFGAGTKLELK

SEQ ID NO: 22 - protein, 11 aa, synthetic construct
KASQDINTYLS

SEQ ID NO: 23 - protein, 7 aa, synthetic construct
RANRLVD

SEQ ID NO: 24 - protein, 9 aa, synthetic construct
LQYDEFPLT

SEQ ID NO: 25 - protein, 117 aa, synthetic construct
EVQLQQSVAELVRPGASVKLSCTASGFNIQNTYMHWVKQRPEQGLEWIGRIDPANGNTKYAPKFQGKATITADTSSNTAYLQLSSLTSEDTAIYYCARYYDSRYGYWGQGTTLTVSS

SEQ ID NO: 26 - protein, 5 aa, synthetic construct
NTYMH

SEQ ID NO: 27 - protein, 17 aa, synthetic construct
RIDPANGNTKYAPKFQG

SEQ ID NO: 28 - protein, 8 aa, synthetic construct
YYDSRYGY

SEQ ID NO: 29 - protein, 107 aa, synthetic construct
DIKMTQSPSSMYASLGERVTITCKASQDINSYLSWFQQKPGKSPTTLIYRANRLVDGVPSRFSGSGSGQDYSLTISSLEYEDLGIYFCLQYDEFPWTFGGGTKLEIK

SEQ ID NO: 30 - protein, 11 aa, synthetic construct
KASQDINSYLS

SEQ ID NO: 31 - protein, 7 aa, synthetic construct
RANRLVD

SEQ ID NO: 32 - protein, 9 aa, synthetic construct
LQYDEFPWT

SEQ ID NO: 33 - protein, 119 aa, synthetic construct
EVQLQQSVAELVRPGASVKLSCTASGFNIKNTYMDWVKQRPEQGLEWIGRIDPANGNTKYAPKFQGKATITADTSSNTAYLQLSSLTSEDTAIYYCAREGNWDDWFVYWGQGTLVTVSA

SEQ ID NO: 34 - protein, 5 aa, synthetic construct
NTYMD

SEQ ID NO: 35 - protein, 17 aa, synthetic construct
RIDPANGNTKYAPKFQG

SEQ ID NO: 36 - protein, 10 aa, synthetic construct
EGNWDDWFVY

SEQ ID NO: 37 - protein, 112 aa, synthetic construct
DVLMTQTPLSLPVSLGDQASISCRSSQSIVHSNGNTYLEWFLQKPGQSPKLLIYKVSNRFSGVPDRFSGSGSGTDFTLKISRVEAEDLGVYYCFQGSHVPPTFGGGTKLEIK

SEQ ID NO: 38 - protein, 16 aa, synthetic construct
RSSQSIVHSNGNTYLE

SEQ ID NO: 39 - protein, 7 aa, synthetic construct
KVSNRFS

SEQ ID NO: 40 - protein, 9 aa, synthetic construct
FQGSHVPPT

SEQ ID NO: 41 - protein, 119 aa, synthetic construct
EVQLQQSVAELVRPGASVKLSCTASGFNIKNTYMDWVKQRPEQGLEWIGRIDPANGNTKHAPKFQGKATITTDTSSNTAYLQLSSLTSEDTAIYYCARWGGWDVRFAYWGQGTLVTVSA

SEQ ID NO: 42 - protein, 5 aa, synthetic construct
NTYMD

SEQ ID NO: 43 - protein, 17 aa, synthetic construct
RIDPANGNTKHAPKFQG

SEQ ID NO: 44 - protein, 10 aa, synthetic construct
WGGWDVRFAY

SEQ ID NO: 45 - protein, 107 aa, synthetic construct
DIKMTQSPSSMYASLGERVTINCQASQDINSYLSWFQQKPGKSPKTLIHRANRLVDGVPSRFSGSGSGQDYSLTISSLEYEDMGIYYCLQFDEFPLTFGAGTKLELK

SEQ ID NO: 46 - protein, 11 aa, synthetic construct
QASQDINSYLS

SEQ ID NO: 47 - protein, 7 aa, synthetic construct
RANRLVD

SEQ ID NO: 48 - protein, 9 aa, synthetic construct
LQFDEFPLT

SEQ ID NO: 49 - protein, 121 aa, synthetic construct
EVQLQQSVAELVRPGASVKLSCTASGFNIQNTYIHWVKQRPEQGLEWIGRIDPASGSTEYAPKFQGKATITADTSSNSGYLQLSSLTSEDTAIYYCARYGNFLYYYSMDYWGQGTSVTVSA

SEQ ID NO: 50 - protein, 5 aa, synthetic construct
NTYIH

SEQ ID NO: 51 - protein, 17 aa, synthetic construct
RIDPASGSTEYAPKFQG

SEQ ID NO: 52 - protein, 12 aa, synthetic construct
YGNFLYYYSMDY

SEQ ID NO: 53 - protein, 112 aa, synthetic construct
DIVMTQAAPSVPVTPGESVSISCRSNKSLLHSNGNTYLYWFLQRPGQSPQLLIYRMSNLASGVPDRFSGSGSGTAFTLRISRVEAEDVGVYYCMQHLENPYTFGGGTKLEIK

SEQ ID NO: 54 - protein, 16 aa, synthetic construct
RSNKSLLHSNGNTYLY

SEQ ID NO: 55 - protein, 7 aa, synthetic construct
RMSNLAS

SEQ ID NO: 56 - protein, 9 aa, synthetic construct
MQHLENPYT

SEQ ID NO: 57 - protein, 120 aa, synthetic construct
EVQLQQSVAELVRPGASVKLSCTASGFNIQNTYLHWVKQRPEQGLEWIGRIDPANDNIKYVPKFQGKATITADTSSNTAYLQLSSLTSEDTAIYYCTRHGLFYEGWFAYWGQGTLVTVST

SEQ ID NO: 58 - protein, 5 aa, synthetic construct
NTYLH

SEQ ID NO: 59 - protein, 17 aa, synthetic construct
RIDPANDNIKYVPKFQG

SEQ ID NO: 60 - protein, 11 aa, synthetic construct
HGLFYEGWFAY

SEQ ID NO: 61 - protein, 108 aa, synthetic construct
EIVLTQSPALMAASPGEKVTITCSVSSSISSSNLHWYQQKSGTSPKPWIYGTSNLASGVPVRFSGSGSGTSYSLTISSMEAEDAATYYCQQWSSYPYTFGSGTKLEIK

SEQ ID NO: 62 - protein, 12 aa, synthetic construct
SVSSSISSSNLH

SEQ ID NO: 63 - protein, 7 aa, synthetic construct
GTSNLAS

SEQ ID NO: 64 - protein, 9 aa, synthetic construct
QQWSSYPYT

SEQ ID NO: 65 - protein, 121 aa, synthetic construct
QVQLVQSGAEVKKPGASVKVSCKASGFNIQNTYIHWVRQAPGQGLEWMGRIDPASGSTEYAPKFQGRVTMTADTSTNTGYMELSSLRSEDTAVYYCARYGNFLYYYSMDYWGQGTLVTVSS

SEQ ID NO: 66 - protein, 112 aa, synthetic construct
DIVMTQSPLSLPVTLGQPASISCRSNKSLLHSNGNTYLYWFQQRPGQSPRLLIYRMSNLASGVPDRFSGSGSGTDFTLKISRVEAEDVGVYYCMQHLENPYTFGQGTKLEIK

SEQ ID NO: 67 - protein, 112 aa, synthetic construct
  MOD_RES 26: note = T,S,Q,A,D,G,E,F,I,K,L,P,V,W,Y,R,H
  MOD_RES 33: note = N,Q,S,T
  MOD_RES 34: note = G,A,L,E,K,R,S,N,T,Q
DIVMTQSPLSLPVTLGQPASISCRSXKSLLHSXXNTYLYWFQQRPGQSPRLLIYRMSNLASGVPDRFSGSGSGTDFTLKISRVEAEDVGVYYCMQHLENPYTFGQGTKLEIK

SEQ ID NO: 68 - protein, 16 aa, synthetic construct
  MOD_RES 3: note = T,S,Q,A,D,G,E,F,I,K,L,P,V,W,Y,R,H
  MOD_RES 10: note = N,Q,S,T
  MOD_RES 11: note = G,A,L,E,K,R,S,N,T,Q
RSXKSLLHSXXNTYLY

SEQ ID NO: 69 - DNA, 363 bp, synthetic construct
  source 1..363: mol_type = other DNA
gaggtacagttgcaacagtctgttgcagagcttgtgaggccaggtgcctctgtcaaactgtcttgtactgccagcgggttcaatatccagaacacatatatgcactgggtaaaggagaggccagagcagggcttggagtggataggaagaatcgacccagccaatggcgacactgagtttgctcctaagttccaggggaaagctaccctcacaacagatacctctagcaacactgcctatctccagctgtcctctctgacctccgaggatactgccatctactattgcggcagagagagatacttctacggaagcagaggcttcgcctattgggggcaaggaacactggttacagtgtctgca

SEQ ID NO: 70 - DNA, 321 bp, synthetic construct
  source 1..321: mol_type = other DNA
gacatattgatgacacagtctcctccctctatgtcagtctcactgggcgatactgtttcaattacatgccacgccagccagggcatttcatcaaacatcggctggttgcagcagaaaccaggcaagtctttcaagggactcatctatcacggcaccaacttggaggatggtgtgccttcccgattctccggatcaggctccggcgccgattactccctgaccatttctagcctggaatccgaggacttcgccgactactattgtgtacagtatgctcagttcccatggacattcggagggggaaccaagctcgaaataaaa

SEQ ID NO: 71 - DNA, 366 bp, synthetic construct
  source 1..366: mol_type = other DNA
gaagtacagcttcaacagtcagtagccgagttggtgagaccaggtgcatcagtgaagttgagctgtactgctagtggtttcaacattaagaacacatatatccactgggtcaaacagaggcccgagcaaggactggagtggataggcaggatcgatccagcaaacggaaataccaaatacgctcctaagtttcaggggaaggcttccattattgtggataccagttctaacacggcctacctgcagctgtccagcctcacctccgaggataccgccatctactactgcgcccgatattatgcctccagcccctattattataatatggattactggggccagggcacttccgttacagtgagctcc

SEQ ID NO: 72 - DNA, 318 bp, synthetic construct
  source 1..318: mol_type = other DNA
gatattcagatgacccagtctccggcaagcctgtcagtgagtgtgggcgagacagtgacaatcacctgtagggccagcgaaaacatctatagcaatctcgcatggtatcaacagaaacagggtaagtcaccacagctgcttgtgtatgctgccaccaacctggccgatggagtcccatccagattttctggctctgggagcgggacacaatactccctcaagattaacagcctccaaagcgaggactttgggtcctactactgccagcacttttggggaacatttacgttcggcagcgggacaaaactcgaaatcaag

SEQ ID NO: 73 - DNA, 357 bp, synthetic construct
  source 1..357: mol_type = other DNA
gaagttcagcttcaacagtctgtggctgaacttgtacgcccaggggcatccgtgaagttgagttgtacagccagcggcttcaatatcaaaaacacctacatcgattgggtgaaacagcgacctgagcagggactggaatggatcggcaacattgacccggctaacggcaacaccaaatacgctccgaaattccagggtaaagctactattacagctgatacctcctccaacaccgcctacgtccagctgagcagcctgacctctgaagatacagctatctactactgtgccaggtggggaggttgggacgtgaggttcgcctattggggacagggaaccctcgtcactgtcagcgct

SEQ ID NO: 74 - DNA, 321 bp, synthetic construct
  source 1..321: mol_type = other DNA
gacatcaagatgacgcagtcaccaagctctatgtacgcctcactgggggagcgagtaaccatcacttgtaaggcatcccaggatatcaacacttacctgagctggtttcagcaaaagcctggcaagtcccccaagaccctcatctatagagctaatcgcctcgtggacggagtgcccagccggtttagtggatccggatccggccagaactattccctgacaatcagcagcctggagtatgaggacatggggatttattactgtctgcaatatgatgagttcccgctcactttcggagccggaaccaagcttgagttgaag

SEQ ID NO: 75 - DNA, 351 bp, synthetic construct
  source 1..351: mol_type = other DNA
gaggtacagctgcagcaatctgttgccgaattggtgagaccaggtgcctcagtgaaactgtcttgcactgcctctggattcaatatccagaatacttacatgcattgggtcaagcagagacccgaacaggggctcgaatggataggaaggattgatcccgctaacggcaacacaaagtacgctccaaaattccaaggaaaagccactataaccgccgatactagcagcaataccgcttatctccagctgtcttccctgacaagtgaggacacggccatttattattgtgccagatattacgatagtaggtacggatattggggacagggaacaacactgacagtgtcctcc

SEQ ID NO: 76 - DNA, 321 bp, synthetic construct
  source 1..321: mol_type = other DNA
gacatcaagatgacacagtccccatctagtatgtacgctagccttggtgagcgggtgacaatcacttgcaaagcctcccaggacatcaactcatacctgtcctggttccagcagaagcccgggaagagtccaaccacactgatataccgagccaaccgactggtagatggcgtgccttctcggttctccggctcaggtagcgggcaggactactccctgactatttcctctctcgaatacgaagatctgggcatctacttctgtctccagtacgacgaatttccctggacgttcggaggaggaaccaagcttgagattaag

SEQ ID NO: 77 - DNA, 357 bp, synthetic construct
  source 1..357: mol_type = other DNA
gaggtgcagttgcagcaaagcgttgcagaacttgttagacctggtgctagtgtgaaactgagctgcaccgccagtggatttaacatcaagaacacctacatggactgggtcaaacagaggcccgagcaggggttggagtggattggacgaattgatcccgcaaacgggaacacaaaatacgctcctaagtttcagggaaaagccaccattacagcagacaccagtagcaataccgcttatctgcagctgtctagcctgaccagcgaggacaccgcaatatactactgcgccagagaagggaattgggatgattggttcgtatactggggacagggcacactggtgacagtctctgct

SEQ ID NO: 78 - DNA, 336 bp, synthetic construct
  source 1..336: mol_type = other DNA
gatgtcctgatgacccagaccccactgagtctcccagtaagtttgggcgaccaggcatcaatctcatgtagaagcagccagtctatcgtgcacagcaacggcaatacatacctcgagtggttcctccagaaaccaggtcagtcccctaagctgctcatctacaaggtcagcaaccggtttagcggtgtaccagacagattctctgggtccggctccggaactgactttacccttaagatctctagggtggaagccgaagatctcggagtgtactactgtttccaggggtcacatgtgccacctacttttggaggcgggactaagttggagataaag

SEQ ID NO: 79 - DNA, 357 bp, synthetic construct
  source 1..357: mol_type = other DNA
gaagtgcaactgcagcaatctgtcgctgaactcgtgagacctggtgcatctgtcaaattgtcatgtacggcatcaggctttaacattaaaaatacatacatggattgggtcaaacagcggccagaacagggtctggaatggatcggaaggattgatccagctaatggtaacaccaagcatgctcccaagtttcagggaaaggccaccattaccactgatacaagcagcaatactgcttacctgcagctgagctccttgaccagcgaggacaccgcaatttattattgtgccaggtggggaggatgggatgtgcgctttgcctactggggccagggtaccctggtaactgtctccgcc

SEQ ID NO: 80 - DNA, 321 bp, synthetic construct
  source 1..321: mol_type = other DNA
gacatcaaaatgactcagagtcctagcagtatgtacgcatctctcggggagcgagttaccatcaactgccaggccagccaagatatcaactcttacctgtcatggttccagcagaagcccggaaagagtccgaagaccttgattcaccgagctaataggctggtggatggcgtgccaagccgcttcagtggtagtggctctggacaggactattcactgaccattagcagcttggaatacgaggatatgggcatctactactgtctgcaatttgacgagttcccactgacattcggcgccggcacaaaacttgagttgaaa

SEQ ID NO: 81 - DNA, 363 bp, synthetic construct
  source 1..363: mol_type = other DNA
gaagtccagcttcagcagtctgttgcagaactggtaagacctggggcctcagtaaagttgagctgcactgctagcggcttcaacatccagaacacctacatccactgggtgaaacagagacccgaacaaggattggagtggattggccgaatagatcccgcctccgggagtactgagtacgctcctaagttccagggcaaggccacaatcacagccgatacctcctctaacagcggttacctgcagctgagcagcttgacctccgaggatactgcaatttactattgtgcaagatacggcaactttctgtattattacagtatggactactggggacagggaacctccgtcactgtgtctgcc

SEQ ID NO: 82 - DNA, 336 bp, synthetic construct
  source 1..336: mol_type = other DNA
gacatcgttatgacacaggctgccccttctgttcccgtaacaccaggggagagcgtgagcattagctgtcggtcaaacaagtctcttctgcacagcaacggaaatacctatctgtactggtttctgcagcgcccaggacagagtccccagcttttgatctacagaatgagtaacttggccagcggggtgccagatcgcttttccggatcaggaagcggcaccgcctttaccctgcggatttctcgggtcgaggcagaggatgtgggggtgtactactgcatgcagcaccttgaaaatccatacactttcgggggaggaaccaagctcgagatcaag

SEQ ID NO: 83 - DNA, 360 bp, synthetic construct
  source 1..360: mol_type = other DNA
gaagtacagcttcaacagagtgttgcagagttggtgcgccctggagcctctgtgaaactgagctgcacagcatccggtttcaacatccagaatacttacctgcattgggtgaagcagcggcctgagcagggtctggagtggattggaagaatcgaccctgcaaatgataatatcaagtatgtgccaaagttccagggcaaggcaaccattacagccgatactagcagcaataccgcctacctgcagctttcaagccttacatctgaggacactgctatctactactgcacaagacacggtctgttctacgaggggtggtttgcttactgggggcaggggacccttgttaccgtgtctaca

SEQ ID NO: 84 - DNA, 324 bp, synthetic construct
  source 1..324: mol_type = other DNA
gaaattgtactgacacagtctccagccttgatggctgcctcccctggtgagaaggtgactattacctgtagcgtgagcagttctatttccagctccaacctgcactggtatcagcagaagagcggcaccagtccaaagccctggatatatggcacctccaaccttgcatccggcgtgcccgtgcgattcagtggctcaggttccggtacttcctactctctcaccatctcctctatggaagccgaagacgcagctacatactactgccagcagtggtccagttacccctacactttcggctctggaaccaagctggaaatcaag

SEQ ID NO: 85 - protein, 121 aa, synthetic construct
QVQLVQSGAEVKKPGASVKVSCKASGFNIQNTYIHWVRQAPGQGLEWIGRIDPASGSTEYAPKFQGRATITADTSTNTGYMELSSLRSEDTAVYYCARYGNFLYYYSMDYWGQGTLVTVSS

SEQ ID NO: 86 - protein, 121 aa, synthetic construct
QVQLVQSGAEVKKPGASVKVSCKASGFNIQNTYIHWVRQAPGQGLEWMGRIDPASGSTEYAPKFQGRVTMTADTSINTGYMELSRLRSDDTAVYYCARYGNFLYYYSMDYWGQGTLVTVSS

SEQ ID NO: 87 - protein, 112 aa, synthetic construct
DIVMTQSPLSLPVTPGEPASISCRSNKSLLHSNGNTYLYWFLQKPGQSPQLLIYRMSNLASGVPDRFSGSGSGTDFTLKISRVEAEDVGVYYCMQHLENPYTFGQGTKLEIK

SEQ ID NO: 88 - protein, 111 aa, synthetic construct
DIVMTQTPLSLSVTPGQPASISCRSNKSLLHSNGNTYLYWFLQKPGQPPQLLIYRMSNLASGVPDRFSGSGSGTDFTLKISRVEAEDVGVYYCMQHLENPYTFGQGTKLEI

SEQ ID NO: 89 - protein, 120 aa, synthetic construct
QVQLVQSGAEVKKPGASVKVSCKASGFNIQNTYLHWVRQAPGQGLEWMGRIDPANDNIKYVPKFQGRVTMTADTSTNTAYMELSSLRSEDTAVYYCTRHGLFYEGWFAYWGQGTLVTVSS

SEQ ID NO: 90 - protein, 120 aa, synthetic construct
QVQLVQSGAEVKKPGASVKVSCKASGFNIQNTYLHWVRQAPGQGLEWMGRIDPANDNIKYVPKFQGRVTMTADTSINTAYMELSRLRSDDTAVYYCTRHGLFYEGWFAYWGQGTLVTVSS

SEQ ID NO: 91 - protein, 120 aa, synthetic construct
QVQLVQSGAEVKKPGSSVKVSCKASGFNIQNTYLHWVRQAPGQGLEWMGRIDPANDNIKYVPKFQGRVTITADTSTNTAYMELSSLRSEDTAVYYCTRHGLFYEGWFAYWGQGTLVTVSS

SEQ ID NO: 92 - protein, 108 aa, synthetic construct
DIQLTQSPSSLSASVGDRVTITCSVSSSISSSNLHWYQQKPGKAPKPLIYGTSNLASGVPSRFSGSGSGTDYTLTISSLQPEDAATYYCQQWSSYPYTFGQGTKLEIK

SEQ ID NO: 93 - protein, 108 aa, synthetic construct
DIQLTQSPSTLSASVGDRVTITCSVSSSISSSNLHWYQQKPGKAPKPLIYGTSNLASGVPSRFSGSGSGTEYTLTISSLQPDDAATYYCQQWSSYPYTFGQGTKLEIK

SEQ ID NO: 94 - protein, 108 aa, synthetic construct
EIVLTQSPATLSLSPGERATLSCSVSSSISSSNLHWYQQKPGQAPRPLIYGTSNLASGIPARFSGSGSGTDYTLTISSLEPEDAAVYYCQQWSSYPYTFGQGTKLEIK

SEQ ID NO: 95 - protein, 327 aa, synthetic construct
ASTKGPSVFPLAPCSRSTSESTAALGCLVKDYFPEPVTVSWNSGALTSGVHTFPAVLQSSGLYSLSSVVTVPSSSLGTKTYTCNVDHKPSNTKVDKRVESKYGPPCPPCPAPEFLGGPSVFLFPPKPKDTLMISRTPEVTCVVVDVSQEDPEVQFNWYVDGVEVHNAKTKPREEQFNSTYRVVSVLTVLHQDWLNGKEYKCKVSNKGLPSSIEKTISKAKGQPREPQVYTLPPSQEEMTKNQVSLTCLVKGFYPSDIAVEWESNGQPENNYKTTPPVLDSDGSFFLYSRLTVDKSRWQEGNVFSCSVMHEALHNHYTQKSLSLSLGK

SEQ ID NO: 96 - protein, 107 aa, synthetic construct [sequence omitted]

SEQ ID NO: 97 - protein, 112 aa, synthetic construct
DIVMTQSPLSLPVTLGQPASISCRSSKSLLHSSGNTYLYWFQQRPGQSPRLLIYRMSNLASGVPDRFSGSGSGTDFTLKISRVEAEDVGVYYCMQHLENPYTFGQGTKLEIK

SEQ ID NO: 98 - protein, 16 aa, synthetic construct
RSSKSLLHSSGNTYLY

SEQ ID NO: 99 - protein, 112 aa, synthetic construct
DIVMTQSPLSLPVTLGQPASISCRSSKSLLHSQGNTYLYWFQQRPGQSPRLLIYRMSNLASGVPDRFSGSGSGTDFTLKISRVEAEDVGVYYCMQHLENPYTFGQGTKLEIK

SEQ ID NO: 100 - protein, 16 aa, synthetic construct
RSSKSLLHSQGNTYLY

SEQ ID NO: 101 - protein, 112 aa, synthetic construct
DIVMTQSPLSLPVTLGQPASISCRSSKSLLHSTGNTYLYWFQQRPGQSPRLLIYRMSNLASGVPDRFSGSGSGTDFTLKISRVEAEDVGVYYCMQHLENPYTFGQGTKLEIK

SEQ ID NO: 102 - protein, 16 aa, synthetic construct
RSSKSLLHSTGNTYLY

SEQ ID NO: 103 - protein, 112 aa, synthetic construct
DIVMTQSPLSLPVTLGQPASISCRSSKSLLHSNANTYLYWFQQRPGQSPRLLIYRMSNLASGVPDRFSGSGSGTDFTLKISRVEAEDVGVYYCMQHLENPYTFGQGTKLEIK

SEQ ID NO: 104 - protein, 16 aa, synthetic construct
RSSKSLLHSNANTYLY

SEQ ID NO: 105 - protein, 112 aa, synthetic construct
DIVMTQSPLSLPVTLGQPASISCRSTKSLLHSSGNTYLYWFQQRPGQSPRLLIYRMSNLASGVPDRFSGSGSGTDFTLKISRVEAEDVGVYYCMQHLENPYTFGQGTKLEIK

SEQ ID NO: 106 - protein, 16 aa, synthetic construct
RSTKSLLHSSGNTYLY

SEQ ID NO: 107 - protein, 112 aa, synthetic construct
DIVMTQSPLSLPVTLGQPASISCRSTKSLLHSQGNTYLYWFQQRPGQSPRLLIYRMSNLASGVPDRFSGSGSGTDFTLKISRVEAEDVGVYYCMQHLENPYTFGQGTKLEIK

SEQ ID NO: 108 - protein, 16 aa, synthetic construct
RSTKSLLHSQGNTYLY

SEQ ID NO: 109 - protein, 112 aa, synthetic construct
DIVMTQSPLSLPVTLGQPASISCRSTKSLLHSTGNTYLYWFQQRPGQSPRLLIYRMSNLASGVPDRFSGSGSGTDFTLKISRVEAEDVGVYYCMQHLENPYTFGQGTKLEIK

SEQ ID NO: 110 - protein, 16 aa, synthetic construct
RSTKSLLHSTGNTYLY

SEQ ID NO: 111 - protein, 112 aa, synthetic construct
DIVMTQSPLSLPVTLGQPASISCRSTKSLLHSNANTYLYWFQQRPGQSPRLLIYRMSNLASGVPDRFSGSGSGTDFTLKISRVEAEDVGVYYCMQHLENPYTFGQGTKLEIK

SEQ ID NO: 112 - protein, 16 aa, synthetic construct
RSTKSLLHSNANTYLY

SEQ ID NO: 113 - protein, 112 aa, synthetic construct
DIVMTQSPLSLPVTLGQPASISCRSAKSLLHSNANTYLYWFQQRPGQSPRLLIYRMSNLASGVPDRFSGSGSGTDFTLKISRVEAEDVGVYYCMQHLENPYTFGQGTKLEIK

SEQ ID NO: 114 - protein, 16 aa, synthetic construct
RSAKSLLHSNANTYLY

SEQ ID NO: 115 - protein, 112 aa, synthetic construct
DIVMTQSPLSLPVTLGQPASISCRSDKSLLHSNANTYLYWFQQRPGQSPRLLIYRMSNLASGVPDRFSGSGSGTDFTLKISRVEAEDVGVYYCMQHLENPYTFGQGTKLEIK

SEQ ID NO: 116 - protein, 16 aa, synthetic construct
RSDKSLLHSNANTYLY

SEQ ID NO: 117 - protein, 112 aa, synthetic construct
DIVMTQSPLSLPVTLGQPASISCRSEKSLLHSNANTYLYWFQQRPGQSPRLLIYRMSNLASGVPDRFSGSGSGTDFTLKISRVEAEDVGVYYCMQHLENPYTFGQGTKLEIK

SEQ ID NO: 118 - protein, 16 aa, synthetic construct
RSEKSLLHSNANTYLY

SEQ ID NO: 119 - protein, 112 aa, synthetic construct
DIVMTQSPLSLPVTLGQPASISCRSFKSLLHSNANTYLYWFQQRPGQSPRLLIYRMSNLASGVPDRFSGSGSGTDFTLKISRVEAEDVGVYYCMQHLENPYTFGQGTKLEIK

SEQ ID NO: 120 - protein, 16 aa, synthetic construct
RSFKSLLHSNANTYLY

SEQ ID NO: 121 - protein, 112 aa, synthetic construct
DIVMTQSPLSLPVTLGQPASISCRSGKSLLHSNANTYLYWFQQRPGQSPRLLIYRMSNLASGVPDRFSGSGSGTDFTLKISRVEAEDVGVYYCMQHLENPYTFGQGTKLEIK

SEQ ID NO: 122 - protein, 16 aa, synthetic construct
RSGKSLLHSNANTYLY

SEQ ID NO: 123 - protein, 112 aa, synthetic construct
DIVMTQSPLSLPVTLGQPASISCRSHKSLLHSNANTYLYWFQQRPGQSPRLLIYRMSNLASGVPDRFSGSGSGTDFTLKISRVEAEDVGVYYCMQHLENPYTFGQGTKLEIK

SEQ ID NO: 124 - protein, 16 aa, synthetic construct
RSHKSLLHSNANTYLY

SEQ ID NO: 125 - protein, 112 aa, synthetic construct
DIVMTQSPLSLPVTLGQPASISCRSIKSLLHSNANTYLYWFQQRPGQSPRLLIYRMSNLASGVPDRFSGSGSGTDFTLKISRVEAEDVGVYYCMQHLENPYTFGQGTKLEIK

SEQ ID NO: 126 - protein, 16 aa, synthetic construct
RSIKSLLHSNANTYLY

SEQ ID NO: 127 - protein, 112 aa, synthetic construct
DIVMTQSPLSLPVTLGQPASISCRSKKSLLHSNANTYLYWFQQRPGQSPRLLIYRMSNLASGVPDRFSGSGSGTDFTLKISRVEAEDVGVYYCMQHLENPYTFGQGTKLEIK

SEQ ID NO: 128 - protein, 16 aa, synthetic construct
RSKKSLLHSNANTYLY

SEQ ID NO: 129 - protein, 112 aa, synthetic construct
DIVMTQSPLSLPVTLGQPASISCRSLKSLLHSNANTYLYWFQQRPGQSPRLLIYRMSNLASGVPDRFSGSGSGTDFTLKISRVEAEDVGVYYCMQHLENPYTFGQGTKLEIK

SEQ ID NO: 130 - protein, 16 aa, synthetic construct
RSLKSLLHSNANTYLY

SEQ ID NO: 131 - protein, 112 aa, synthetic construct
DIVMTQSPLSLPVTLGQPASISCRSPKSLLHSNANTYLYWFQQRPGQSPRLLIYRMSNLASGVPDRFSGSGSGTDFTLKISRVEAEDVGVYYCMQHLENPYTFGQGTKLEIK

SEQ ID NO: 132 - protein, 16 aa, synthetic construct
RSPKSLLHSNANTYLY

SEQ ID NO: 133 - protein, 112 aa, synthetic construct
DIVMTQSPLSLPVTLGQPASISCRSQKSLLHSNANTYLYWFQQRPGQSPRLLIYRMSNLASGVPDRFSGSGSGTDFTLKISRVEAEDVGVYYCMQHLENPYTFGQGTKLEIK

SEQ ID NO: 134 - protein, 16 aa, synthetic construct
RSQKSLLHSNANTYLY

SEQ ID NO: 135 - protein, 112 aa, synthetic construct
DIVMTQSPLSLPVTLGQPASISCRSRKSLLHSNANTYLYWFQQRPGQSPRLLIYRMSNLASGVPDRFSGSGSGTDFTLKISRVEAEDVGVYYCMQHLENPYTFGQGTKLEIK

SEQ ID NO: 136 - protein, 16 aa, synthetic construct
RSRKSLLHSNANTYLY

SEQ ID NO: 137 - protein, 112 aa, synthetic construct
DIVMTQSPLSLPVTLGQPASISCRSVKSLLHSNANTYLYWFQQRPGQSPRLLIYRMSNLASGVPDRFSGSGSGTDFTLKISRVEAEDVGVYYCMQHLENPYTFGQGTKLEIK

SEQ ID NO: 138 - protein, 16 aa, synthetic construct
RSVKSLLHSNANTYLY

SEQ ID NO: 139 - protein, 112 aa, synthetic construct
DIVMTQSPLSLPVTLGQPASISCRSWKSLLHSNANTYLYWFQQRPGQSPRLLIYRMSNLASGVPDRFSGSGSGTDFTLKISRVEAEDVGVYYCMQHLENPYTFGQGTKLEIK

SEQ ID NO: 140 - protein, 16 aa, synthetic construct
RSWKSLLHSNANTYLY

SEQ ID NO: 141 - protein, 112 aa, synthetic construct
DIVMTQSPLSLPVTLGQPASISCRSYKSLLHSNANTYLYWFQQRPGQSPRLLIYRMSNLASGVPDRFSGSGSGTDFTLKISRVEAEDVGVYYCMQHLENPYTFGQGTKLEIK

SEQ ID NO: 142 - protein, 16 aa, synthetic construct
RSYKSLLHSNANTYLY

SEQ ID NO: 143 - protein, 112 aa, synthetic construct
DIVMTQSPLSLPVTLGQPASISCRSSKSLLHSNENTYLYWFQQRPGQSPRLLIYRMSNLASGVPDRFSGSGSGTDFTLKISRVEAEDVGVYYCMQHLENPYTFGQGTKLEIK

SEQ ID NO: 144 - protein, 16 aa, synthetic construct
RSSKSLLHSNENTYLY

SEQ ID NO: 145 - protein, 112 aa, synthetic construct
DIVMTQSPLSLPVTLGQPASISCRSSKSLLHSNGNTYLYWFQQRPGQSPRLLIYRMSNLASGVPDRFSGSGSGTDFTLKISRVEAEDVGVYYCMQHLENPYTFGQGTKLEIK

SEQ ID NO: 146 - protein, 16 aa, synthetic construct
RSSKSLLHSNGNTYLY

SEQ ID NO: 147 - protein, 112 aa, synthetic construct
DIVMTQSPLSLPVTLGQPASISCRSSKSLLHSNKNTYLYWFQQRPGQSPRLLIYRMSNLASGVPDRFSGSGSGTDFTLKISRVEAEDVGVYYCMQHLENPYTFGQGTKLEIK

SEQ ID NO: 148 - protein, 16 aa, synthetic construct
RSSKSLLHSNKNTYLY

SEQ ID NO: 149 - protein, 112 aa, synthetic construct
DIVMTQSPLSLPVTLGQPASISCRSSKSLLHSNLNTYLYWFQQRPGQSPRLLIYRMSNLASGVPDRFSGSGSGTDFTLKISRVEAEDVGVYYCMQHLENPYTFGQGTKLEIK

SEQ ID NO: 150 - protein, 16 aa, synthetic construct
RSSKSLLHSNLNTYLY

SEQ ID NO: 151 - protein, 112 aa, synthetic construct
DIVMTQSPLSLPVTLGQPASISCRSSKSLLHSNNNTYLYWFQQRPGQSPRLLIYRMSNLASGVPDRFSGSGSGTDFTLKISRVEAEDVGVYYCMQHLENPYTFGQGTKLEIK

SEQ ID NO: 152 - protein, 16 aa, synthetic construct
RSSKSLLHSNNNTYLY

SEQ ID NO: 153 - protein, 112 aa, synthetic construct
DIVMTQSPLSLPVTLGQPASISCRSSKSLLHSNQNTYLYWFQQRPGQSPRLLIYRMSNLASGVPDRFSGSGSGTDFTLKISRVEAEDVGVYYCMQHLENPYTFGQGTKLEIK

SEQ ID NO: 154 - protein, 16 aa, synthetic construct
RSSKSLLHSNQNTYLY

SEQ ID NO: 155 - protein, 112 aa, synthetic construct
DIVMTQSPLSLPVTLGQPASISCRSSKSLLHSNRNTYLYWFQQRPGQSPRLLIYRMSNLASGVPDRFSGSGSGTDFTLKISRVEAEDVGVYYCMQHLENPYTFGQGTKLEIK

SEQ ID NO: 156 - protein, 16 aa, synthetic construct
RSSKSLLHSNRNTYLY

SEQ ID NO: 157 - protein, 112 aa, synthetic construct
DIVMTQSPLSLPVTLGQPASISCRSSKSLLHSNSNTYLYWFQQRPGQSPRLLIYRMSNLASGVPDRFSGSGSGTDFTLKISRVEAEDVGVYYCMQHLENPYTFGQGTKLEIK

SEQ ID NO: 158 - protein, 16 aa, synthetic construct
RSSKSLLHSNSNTYLY

SEQ ID NO: 159 - protein, 112 aa, synthetic construct
DIVMTQSPLSLPVTLGQPASISCRSSKSLLHSNTNTYLYWFQQRPGQSPRLLIYRMSNLASGVPDRFSGSGSGTDFTLKISRVEAEDVGVYYCMQHLENPYTFGQGTKLEIK

SEQ ID NO: 160 - protein, 16 aa, synthetic construct
RSSKSLLHSNTNTYLY

SEQ ID NO: 161 - protein, 327 aa, synthetic construct
ASTKGPSVFPLAPCSRSTSESTAALGCLVKDYFPEPVTVSWNSGALTSGVHTFPAVLQSSGLYSLSSVVTVPSSSLGTKTYTCNVDHKPSNTKVDKRVESKYGPPCPPCPAPEFEGGPSVFLFPPKPKDTLMISRTPEVTCVVVAVSQEDPEVQFNWYVDGVEVHNAKTKPREEQFNSTYRVVSVLTVLHQDWLNGKEYKCKVSNKGLPSSIEKTISKAKGQPREPQVYTLPPSQEEMTKNQVSLTCLVKGFYPSDIAVEWESNGQPENNYKTTPPVLDSDGSFFLYSKLTVDKSRWQEGNVFSCSVMHEALHNHYTQKSLSLSLGK

SEQ ID NO: 162 - protein, 448 aa, synthetic construct
QVQLVQSGAEVKKPGASVKVSCKASGFNIQNTYIHWVRQAPGQGLEWMGRIDPASGSTEYAPKFQGRVTMTADTSTNTGYMELSSLRSEDTAVYYCARYGNFLYYYSMDYWGQGTLVTVSSASTKGPSVFPLAPCSRSTSESTAALGCLVKDYFPEPVTVSWNSGALTSGVHTFPAVLQSSGLYSLSSVVTVPSSSLGTKTYTCNVDHKPSNTKVDKRVESKYGPPCPPCPAPEFEGGPSVFLFPPKPKDTLMISRTPEVTCVVVAVSQEDPEVQFNWYVDGVEVHNAKTKPREEQFNSTYRVVSVLTVLHQDWLNGKEYKCKVSNKGLPSSIEKTISKAKGQPREPQVYTLPPSQEEMTKNQVSLTCLVKGFYPSDIAVEWESNGQPENNYKTTPPVLDSDGSFFLYSKLTVDKSRWQEGNVFSCSVMHEALHNHYTQKSLSLSLGK

SEQ ID NO: 163 - protein, 219 aa, synthetic construct
DIVMTQSPLSLPVTLGQPASISCRSSKSLLHSNANTYLYWFQQRPGQSPRLLIYRMSNLASGVPDRFSGSGSGTDFTLKISRVEAEDVGVYYCMQHLENPYTFGQGTKLEIKRTVAAPSVFIFPPSDEQLKSGTASVVCLLNNFYPREAKVQWKVDNALQSGNSQESVTEQDSKDSTYSLSSTLTLSKADYEKHKVYACEVTHQGLSSPVTKSFNRGEC

SEQ ID NO: 164 - protein, 447 aa, synthetic construct
QVQLVQSGAEVKKPGSSVKVSCKASGFNIQNTYLHWVRQAPGQGLEWMGRIDPANDNIKYVPKFQGRVTITADTSTNTAYMELSSLRSEDTAVYYCTRHGLFYEGWFAYWGQGTLVTVSSASTKGPSVFPLAPCSRSTSESTAALGCLVKDYFPEPVTVSWNSGALTSGVHTFPAVLQSSGLYSLSSVVTVPSSSLGTKTYTCNVDHKPSNTKVDKRVESKYGPPCPPCPAPEFEGGPSVFLFPPKPKDTLMISRTPEVTCVVVAVSQEDPEVQFNWYVDGVEVHNAKTKPREEQFNSTYRVVSVLTVLHQDWLNGKEYKCKVSNKGLPSSIEKTISKAKGQPREPQVYTLPPSQEEMTKNQVSLTCLVKGFYPSDIAVEWESNGQPENNYKTTPPVLDSDGSFFLYSKLTVDKSRWQEGNVFSCSVMHEALHNHYTQKSLSLSLGK

SEQ ID NO: 165 - protein, 215 aa, synthetic construct
DIQLTQSPSSLSASVGDRVTITCSVSSSISSSNLHWYQQKPGKAPKPLIYGTSNLASGVPSRFSGSGSGTDYTLTISSLQPEDAATYYCQQWSSYPYTFGQGTKLEIKRTVAAPSVFIFPPSDEQLKSGTASVVCLLNNFYPREAKVQWKVDNALQSGNSQESVTEQDSKDSTYSLSSTLTLSKADYEKHKVYACEVTHQGLSSPVTKSFNRGEC

SEQ ID NO: 166 - protein, 448 aa, synthetic construct
QVQLVQSGAEVKKPGASVKVSCKASGFNIQNTYIHWVRQAPGQGLEWMGRIDPASGSTEYAPKFQGRVTMTADTSTNTGYMELSSLRSEDTAVYYCARYGNFLYYYSMDYWGQGTLVTVSSASTKGPSVFPLAPCSRSTSESTAALGCLVKDYFPEPVTVSWNSGALTSGVHTFPAVLQSSGLYSLSSVVTVPSSSLGTKTYTCNVDHKPSNTKVDKRVESKYGPPCPPCPAPEFLGGPSVFLFPPKPKDTLMISRTPEVTCVVVDVSQEDPEVQFNWYVDGVEVHNAKTKPREEQFNSTYRVVSVLTVLHQDWLNGKEYKCKVSNKGLPSSIEKTISKAKGQPREPQVYTLPPSQEEMTKNQVSLTCLVKGFYPSDIAVEWESNGQPENNYKTTPPVLDSDGSFFLYSRLTVDKSRWQEGNVFSCSVMHEALHNHYTQKSLSLSLGK

SEQ ID NO: 167 - protein, 447 aa, synthetic construct
QVQLVQSGAEVKKPGSSVKVSCKASGFNIQNTYLHWVRQAPGQGLEWMGRIDPANDNIKYVPKFQGRVTITADTSTNTAYMELSSLRSEDTAVYYCTRHGLFYEGWFAYWGQGTLVTVSSASTKGPSVFPLAPCSRSTSESTAALGCLVKDYFPEPVTVSWNSGALTSGVHTFPAVLQSSGLYSLSSVVTVPSSSLGTKTYTCNVDHKPSNTKVDKRVESKYGPPCPPCPAPEFLGGPSVFLFPPKPKDTLMISRTPEVTCVVVDVSQEDPEVQFNWYVDGVEVHNAKTKPREEQFNSTYRVVSVLTVLHQDWLNGKEYKCKVSNKGLPSSIEKTISKAKGQPREPQVYTLPPSQEEMTKNQVSLTCLVKGFYPSDIAVEWESNGQPENNYKTTPPVLDSDGSFFLYSRLTVDKSRWQEGNVFSCSVMHEALHNHYTQKSLSLSLGK